European Patent Specification EP 3 791 887 B1, published October 23, 2024. Title: BLOOD PRODUCT DERIVED FROM GENE KNOCKOUT PIG AND USE THEREOF. Applicant: Gcreatene (Suzhou) Biotechnology Co., Ltd. Application WO2019CN85773. The sequence listing filed with the application follows.

SEQUENCE LISTING (21 sequences)

SEQ ID NO: 1 - DNA, 18 bp, Artificial Sequence
  SgRNA nucleotide sequence targeting GGTA1 gene
gaaaataatgaatgtcaa

SEQ ID NO: 2 - DNA, 20 bp, Artificial Sequence
  SgRNA nucleotide sequence targeting CMAH gene
gagtaaggtacgtgatctgt

SEQ ID NO: 3 - DNA, 20 bp, Artificial Sequence
  SgRNA nucleotide sequence targeting Beta-1,4-N-acetyl galactosaminyl transferase 2 gene
ggtagtactcacgaacactc

SEQ ID NO: 4 - DNA, 8505 bp, Artificial Sequence
  Nucleotide sequence of GGTA1-CRISPR/Cas9 vector
tgaccaaaatcccttaacgtgagttttcgttccactgagcgtcagaccccgtagaaaagatcaaaggatcttcttgagatcctttttttctgcgcgtaatctgctgcttgcaaacaaaaaaaccaccgctaccagcggtggtttgtttgccggatcaagagctaccaactctttttccgaaggtaactggcttcagcagagcgcagataccaaatactgtccttctagtgtagccgtagttaggccaccacttcaagaactctgtagcaccgcctacatacctcgctctgctaatcctgttaccagtggctgctgccagtggcgataagtcgtgtcttaccgggttggactcaagacgatagttaccggataaggcgcagcggtcgggctgaacggggggttcgtgcacacagcccagcttggagcgaacgacctacaccgaactgagatacctacagcgtgagctatgagaaagcgccacgcttcccgaagggagaaaggcggacaggtatccggtaagcggcagggtcggaacaggagagcgcacgagggagcttccagggggaaacgcctggtatctttatagtcctgtcgggtttcgccacctctgacttgagcgtcgatttttgtgatgctcgtcaggggggcggagcctatggaaaaacgccagcaacgcggcctttttacggttcctggccttttgctggccttttgctcacatgtgagggcctatttcccatgattccttcatatttgcatatacgatacaaggctgttagagagataattggaattaatttgactgtaaacacaaagatattagtacaaaatacgtgacgtagaaagtaataatttcttgggtagtttgcagttttaaaattatgttttaaaatggactatcatatgcttaccgtaacttgaaagtatttcgatttcttggctttatatatcttgtggaaaggacgaaacaccgaaaataatgaatgtcaagttttagagctagaaatagcaagttaaaataaggctagtccgttatcaacttgaaaaagtggcaccgagtcggtgcttttttgttttagagctagaaatagcaagttaaaataaggctagtccgtttttagcgcgtgcgccaattctgcagacaaatggctctagaggtacccgttacataacttacggtaaatggcccgcctggctgaccgcccaacgacccccgcccattgacgtcaatagtaacgccaatagggactttccattgacgtcaatgggtggagtatttacggtaaactgcccacttggcagtacatcaagtgtatcatatgccaagtacgccccctattgacgtcaatgacggtaaatggcccgcctggcattgtgcccagtacatgaccttatgggactttcctacttggcagtacatctacgtattagtcatcgctattaccatggtcgaggtgagccccacgttctgcttcactctccccatctcccccccctccccacccccaattttgtatttatttattttttaattattttgtgcagcgatgggggcggggggggggggggggcgcgcgccaggcggggcggggcggggcgaggggcggggcggggcgaggcggagaggtgcggcggcagccaatcagagcggcgcgctccgaaagtttccttttatggcgaggcggcggcggcggcggccctataaaaagcgaagcgcgcggcgggcgggagtcgctgcgacgctgccttcgccccgtgccccgctccgccgccgcctcgcgccgcccgccccggctctgactgaccgcgttactcccacaggtgagcgggcgggacggcccttctcctccgggctgtaattagctgagcaagaggtaagggtttaagggatggttggttggtggggtattaatgtttaattacctggagcacctgcctgaaatcactttttttcaggttggaccggtgccaccatggactataaggaccacgacggagactacaaggatcatgatattgattacaaagacgatgacgataagatggccccaaagaagaagcggaaggtcggtatccacggagtcccagcagccgacaagaagtacagcatcggcctggacatcggcaccaactctgtgggctgggccgtgatcaccgacgagtacaaggtgcccagcaagaaattcaaggtgctgggcaacaccgaccggcacagcatcaagaagaacctgatcggagccctgctgttcgacagcggcgaaacagccgaggccacccggctgaagagaaccgccagaagaagatacaccagacggaagaaccggatctgctatctgcaagagatcttcagcaacgagatggccaaggtggacgacagcttcttccacagactggaagagtccttcctggtggaagaggataagaagcacgagcggcaccccatcttcggcaacatcgtggacgaggtggcctaccacgagaagtaccccaccatctaccacctgagaaagaaactggtggacagcaccgacaaggccgacctgcggctgatctatctggccctggcccacatgatcaagttccggggccacttcctgatcgagggcgacctgaaccccgacaacagcgacgtggacaagctgttcatccagctggtgcagacctacaaccagctgttcgaggaaaaccccatcaacgccagcggcgtggacgccaaggccatcctgtctgccagactgagcaagagcagacggctggaaaatctgatcgcccagctgcccggcgagaagaagaatggcctgttcggaaacctgattgccctgagcctgggcctgacccccaacttcaagagcaacttcgacctggccgaggatgccaaactgcagctgagcaaggacacctacgacgacgacctggacaacctgctggcccagatcggcgaccagtacgccgacctgtttctggccgccaagaacctgtccgacgccatcctgctgagcgacatcctgagagtgaacaccgagatcaccaaggcccccctgagcgcctctatgatcaagagatacgacgagcaccaccaggacctgaccctgctgaaagctctcgtgcggcagcagctgcctgagaagtacaaagagattttcttcgaccagagcaagaacggctacgccggctacattgacggcggagccagccaggaagagttctacaagttcatcaagcccatcctggaaaagatggacggcaccgaggaactgctcgtgaagctgaacagagaggacctgctgcggaagcagcggaccttcgacaacggcagcatcccccaccagatccacctgggagagctgcacgccattctgcggcggcaggaagatttttacccattcctgaaggacaaccgggaaaagatcgagaagatcctgaccttccgcatcccctactacgtgggccctctggccaggggaaacagcagattcgcctggatgaccagaaagagcgaggaaaccatcaccccctggaacttcgaggaagtggtggacaagggcgcttccgcccagagcttcatcgagcggatgaccaacttcgataagaacctgcccaacgagaaggtgctgcccaagcacagcctgctgtacgagtacttcaccgtgtataacgagctgaccaaagtgaaatacgtgaccgagggaatgagaaagcccgccttcctgagcggcgagcagaaaaaggccatcgtggacctgctgttcaagaccaaccggaaagtgaccgtgaagcagctgaaagaggactacttcaagaaaatcgagtgcttcgactccgtggaaatctccggcgtggaagatcggttcaacgcctccctgggcacataccacgatctgctgaaaattatcaaggacaaggacttcctggacaatgaggaaaacgaggacattctggaagatatcgtgctgaccctgacactgtttgaggacagagagatgatcgaggaacggctgaaaacctatgcccacctgttcgacgacaaagtgatgaagcagctgaagcggcggagatacaccggctggggcaggctgagccggaagctgatcaacggcatccgggacaagcagtccggcaagacaatcctggatttcctgaagtccgacggcttcgccaacagaaacttcatgcagctgatccacgacgacagcctgacctttaaagaggacatccagaaagcccaggtgtccggccagggcgatagcctgcacgagcacattgccaatctggccggcagccccgccattaagaagggcatcctgcagacagtgaaggtggtggacgagctcgtgaaagtgatgggccggcacaagcccgagaacatcgtgatcgaaatggccagagagaaccagaccacccagaagggacagaagaacagccgcgagagaatgaagcggatcgaagagggcatcaaagagctgggcagccagatcctgaaagaacaccccgtggaaaacacccagctgcagaacgagaagctgtacctgtactacctgcagaatgggcgggatatgtacgtggaccaggaactggacatcaaccggctgtccgactacgatgtggaccatatcgtgcctcagagctttctgaaggacgactccatcgacaacaaggtgctgaccagaagcgacaagaaccggggcaagagcgacaacgtgccctccgaagaggtcgtgaagaagatgaagaactactggcggcagctgctgaacgccaagctgattacccagagaaagttcgacaatctgaccaaggccgagagaggcggcctgagcgaactggataaggccggcttcatcaagagacagctggtggaaacccggcagatcacaaagcacgtggcacagatcctggactcccggatgaacactaagtacgacgagaatgacaagctgatccgggaagtgaaagtgatcaccctgaagtccaagctggtgtccgatttccggaaggatttccagttttacaaagtgcgcgagatcaacaactaccaccacgcccacgacgcctacctgaacgccgtcgtgggaaccgccctgatcaaaaagtaccctaagctggaaagcgagttcgtgtacggcgactacaaggtgtacgacgtgcggaagatgatcgccaagagcgagcaggaaatcggcaaggctaccgccaagtacttcttctacagcaacatcatgaactttttcaagaccgagattaccctggccaacggcgagatccggaagcggcctctgatcgagacaaacggcgaaaccggggagatcgtgtgggataagggccgggattttgccaccgtgcggaaagtgctgagcatgccccaagtgaatatcgtgaaaaagaccgaggtgcagacaggcggcttcagcaaagagtctatcctgcccaagaggaacagcgataagctgatcgccagaaagaaggactgggaccctaagaagtacggcggcttcgacagccccaccgtggcctattctgtgctggtggtggccaaagtggaaaagggcaagtccaagaaactgaagagtgtgaaagagctgctggggatcaccatcatggaaagaagcagcttcgagaagaatcccatcgactttctggaagccaagggctacaaagaagtgaaaaaggacctgatcatcaagctgcctaagtactccctgttcgagctggaaaacggccggaagagaatgctggcctctgccggcgaactgcagaagggaaacgaactggccctgccctccaaatatgtgaacttcctgtacctggccagccactatgagaagctgaagggctcccccgaggataatgagcagaaacagctgtttgtggaacagcacaagcactacctggacgagatcatcgagcagatcagcgagttctccaagagagtgatcctggccgacgctaatctggacaaagtgctgtccgcctacaacaagcaccgggataagcccatcagagagcaggccgagaatatcatccacctgtttaccctgaccaatctgggagcccctgccgccttcaagtactttgacaccaccatcgaccggaagaggtacaccagcaccaaagaggtgctggacgccaccctgatccaccagagcatcaccggcctgtacgagacacggatcgacctgtctcagctgggaggcgacaaaaggccggcggccacgaaaaaggccggccaggcaaaaaagaaaaagtaagaattcctagagctcgctgatcagcctcgactgtgccttctagttgccagccatctgttgtttgcccctcccccgtgccttccttgaccctggaaggtgccactcccactgtcctttcctaataaaatgaggaaattgcatcgcattgtctgagtaggtgtcattctattctggggggtggggtggggcaggacagcaagggggaggattgggaagagaatagcaggcatgctggggagcggccgcaggaacccctagtgatggagttggccactccctctctgcgcgctcgctcgctcactgaggccgggcgaccaaaggtcgcccgacgcccgggctttgcccgggcggcctcagtgagcgagcgagcgcgcagctgcctgcaggggcgcctgatgcggtattttctccttacgcatctgtgcggtatttcacaccgcatacgtcaaagcaaccatagtacgcgccctgtagcggcgcattaagcgcggcgggtgtggtggttacgcgcagcgtgaccgctacacttgccagcgccctagcgcccgctcctttcgctttcttcccttcctttctcgccacgttcgccggctttccccgtcaagctctaaatcgggggctccctttagggttccgatttagtgctttacggcacctcgaccccaaaaaacttgatttgggtgatggttcacgtagtgggccatcgccctgatagacggtttttcgccctttgacgttggagtccacgttctttaatagtggactcttgttccaaactggaacaacactcaaccctatctcgggctattcttttgatttataagggattttgccgatttcggcctattggttaaaaaatgagctgatttaacaaaaatttaacgcgaattttaacaaaatattaacgtttacaattttatggtgcactctcagtacaatctgctctgatgccgcatagttaagccagccccgacacccgccaacacccgctgacgcgccctgacgggcttgtctgctcccggcatccgcttacagacaagctgtgaccgtctccgggagctgcatgtgtcagaggttttcaccgtcatcaccgaaacgcgcgagacgaaagggcctcgtgatacgcctatttttataggttaatgtcatgataataatggtttcttagacgtcaggtggcacttttcggggaaatgtgcgcggaacccctatttgtttatttttctaaatacattcaaatatgtatccgctcatgagacaataaccctgataaatgcttcaataatattgaaaaaggaagagtatgagtattcaacatttccgtgtcgcccttattcccttttttgcggcattttgccttcctgtttttgctcacccagaaacgctggtgaaagtaaaagatgctgaagatcagttgggtgcacgagtgggttacatcgaactggatctcaacagcggtaagatccttgagagttttcgccccgaagaacgttttccaatgatgagcacttttaaagttctgctatgtggcgcggtattatcccgtattgacgccgggcaagagcaactcggtcgccgcatacactattctcagaatgacttggttgagtactcaccagtcacagaaaagcatcttacggatggcatgacagtaagagaattatgcagtgctgccataaccatgagtgataacactgcggccaacttacttctgacaacgatcggaggaccgaaggagctaaccgcttttttgcacaacatgggggatcatgtaactcgccttgatcgttgggaaccggagctgaatgaagccataccaaacgacgagcgtgacaccacgatgcctgtagcaatggcaacaacgttgcgcaaactattaactggcgaactacttactctagcttcccggcaacaattaatagactggatggaggcggataaagttgcaggaccacttctgcgctcggcccttccggctggctggtttattgctgataaatctggagccggtgagcgtggaagccgcggtatcattgcagcactggggccagatggtaagccctcccgtatcgtagttatctacacgacggggagtcaggcaactatggatgaacgaaatagacagatcgctgagataggtgcctcactgattaagcattggtaactgtcagaccaagtttactcatatatactttagattgatttaaaacttcatttttaatttaaaaggatctaggtgaagatcctttttgataatctc

SEQ ID NO: 5 - DNA, 8508 bp, Artificial Sequence
  Nucleotide sequence of CMAH-CRISPR/Cas9 vector
atgaccaaaatcccttaacgtgagttttcgttccactgagcgtcagaccccgtagaaaagatcaaaggatcttcttgagatcctttttttctgcgcgtaatctgctgcttgcaaacaaaaaaaccaccgctaccagcggtggtttgtttgccggatcaagagctaccaactctttttccgaaggtaactggcttcagcagagcgcagataccaaatactgtccttctagtgtagccgtagttaggccaccacttcaagaactctgtagcaccgcctacatacctcgctctgctaatcctgttaccagtggctgctgccagtggcgataagtcgtgtcttaccgggttggactcaagacgatagttaccggataaggcgcagcggtcgggctgaacggggggttcgtgcacacagcccagcttggagcgaacgacctacaccgaactgagatacctacagcgtgagctatgagaaagcgccacgcttcccgaagggagaaaggcggacaggtatccggtaagcggcagggtcggaacaggagagcgcacgagggagcttccagggggaaacgcctggtatctttatagtcctgtcgggtttcgccacctctgacttgagcgtcgatttttgtgatgctcgtcaggggggcggagcctatggaaaaacgccagcaacgcggcctttttacggttcctggccttttgctggccttttgctcacatgtgagggcctatttcccatgattccttcatatttgcatatacgatacaaggctgttagagagataattggaattaatttgactgtaaacacaaagatattagtacaaaatacgtgacgtagaaagtaataatttcttgggtagtttgcagttttaaaattatgttttaaaatggactatcatatgcttaccgtaacttgaaagtatttcgatttcttggctttatatatcttgtggaaaggacgaaacaccgagtaaggtacgtgatctgtgttttagagctagaaatagcaagttaaaataaggctagtccgttatcaacttgaaaaagtggcaccgagtcggtgcttttttgttttagagctagaaatagcaagttaaaataaggctagtccgtttttagcgcgtgcgccaattctgcagacaaatggctctagaggtacccgttacataacttacggtaaatggcccgcctggctgaccgcccaacgacccccgcccattgacgtcaatagtaacgccaatagggactttccattgacgtcaatgggtggagtatttacggtaaactgcccacttggcagtacatcaagtgtatcatatgccaagtacgccccctattgacgtcaatgacggtaaatggcccgcctggcattgtgcccagtacatgaccttatgggactttcctacttggcagtacatctacgtattagtcatcgctattaccatggtcgaggtgagccccacgttctgcttcactctccccatctcccccccctccccacccccaattttgtatttatttattttttaattattttgtgcagcgatgggggcggggggggggggggggcgcgcgccaggcggggcggggcggggcgaggggcggggcggggcgaggcggagaggtgcggcggcagccaatcagagcggcgcgctccgaaagtttccttttatggcgaggcggcggcggcggcggccctataaaaagcgaagcgcgcggcgggcgggagtcgctgcgacgctgccttcgccccgtgccccgctccgccgccgcctcgcgccgcccgccccggctctgactgaccgcgttactcccacaggtgagcgggcgggacggcccttctcctccgggctgtaattagctgagcaagaggtaagggtttaagggatggttggttggtggggtattaatgtttaattacctggagcacctgcctgaaatcactttttttcaggttggaccggtgccaccatggactataaggaccacgacggagactacaaggatcatgatattgattacaaagacgatgacgataagatggccccaaagaagaagcggaaggtcggtatccacggagtcccagcagccgacaagaagtacagcatcggcctggacatcggcaccaactctgtgggctgggccgtgatcaccgacgagtacaaggtgcccagcaagaaattcaaggtgctgggcaacaccgaccggcacagcatcaagaagaacctgatcggagccctgctgttcgacagcggcgaaacagccgaggccacccggctgaagagaaccgccagaagaagatacaccagacggaagaaccggatctgctatctgcaagagatcttcagcaacgagatggccaaggtggacgacagcttcttccacagactggaagagtccttcctggtggaagaggataagaagcacgagcggcaccccatcttcggcaacatcgtggacgaggtggcctaccacgagaagtaccccaccatctaccacctgagaaagaaactggtggacagcaccgacaaggccgacctgcggctgatctatctggccctggcccacatgatcaagttccggggccacttcctgatcgagggcgacctgaaccccgacaacagcgacgtggacaagctgttcatccagctggtgcagacctacaaccagctgttcgaggaaaaccccatcaacgccagcggcgtggacgccaaggccatcctgtctgccagactgagcaagagcagacggctggaaaatctgatcgcccagctgcccggcgagaagaagaatggcctgttcggaaacctgattgccctgagcctgggcctgacccccaacttcaagagcaacttcgacctggccgaggatgccaaactgcagctgagcaaggacacctacgacgacgacctggacaacctgctggcccagatcggcgaccagtacgccgacctgtttctggccgccaagaacctgtccgacgccatcctgctgagcgacatcctgagagtgaacaccgagatcaccaaggcccccctgagcgcctctatgatcaagagatacgacgagcaccaccaggacctgaccctgctgaaagctctcgtgcggcagcagctgcctgagaagtacaaagagattttcttcgaccagagcaagaacggctacgccggctacattgacggcggagccagccaggaagagttctacaagttcatcaagcccatcctggaaaagatggacggcaccgaggaactgctcgtgaagctgaacagagaggacctgctgcggaagcagcggaccttcgacaacggcagcatcccccaccagatccacctgggagagctgcacgccattctgcggcggcaggaagatttttacccattcctgaaggacaaccgggaaaagatcgagaagatcctgaccttccgcatcccctactacgtgggccctctggccaggggaaacagcagattcgcctggatgaccagaaagagcgaggaaaccatcaccccctggaacttcgaggaagtggtggacaagggcgcttccgcccagagcttcatcgagcggatgaccaacttcgataagaacctgcccaacgagaaggtgctgcccaagcacagcctgctgtacgagtacttcaccgtgtataacgagctgaccaaagtgaaatacgtgaccgagggaatgagaaagcccgccttcctgagcggcgagcagaaaaaggccatcgtggacctgctgttcaagaccaaccggaaagtgaccgtgaagcagctgaaagaggactacttcaagaaaatcgagtgcttcgactccgtggaaatctccggcgtggaagatcggttcaacgcctccctgggcacataccacgatctgctgaaaattatcaaggacaaggacttcctggacaatgaggaaaacgaggacattctggaagatatcgtgctgaccctgacactgtttgaggacagagagatgatcgaggaacggctgaaaacctatgcccacctgttcgacgacaaagtgatgaagcagctgaagcggcggagatacaccggctggggcaggctgagccggaagctgatcaacggcatccgggacaagcagtccggcaagacaatcctggatttcctgaagtccgacggcttcgccaacagaaacttcatgcagctgatccacgacgacagcctgacctttaaagaggacatccagaaagcccaggtgtccggccagggcgatagcctgcacgagcacattgccaatctggccggcagccccgccattaagaagggcatcctgcagacagtgaaggtggtggacgagctcgtgaaagtgatgggccggcacaagcccgagaacatcgtgatcgaaatggccagagagaaccagaccacccagaagggacagaagaacagccgcgagagaatgaagcggatcgaagagggcatcaaagagctgggcagccagatcctgaaagaacaccccgtggaaaacacccagctgcagaacgagaagctgtacctgtactacctgcagaatgggcgggatatgtacgtggaccaggaactggacatcaaccggctgtccgactacgatgtggaccatatcgtgcctcagagctttctgaaggacgactccatcgacaacaaggtgctgaccagaagcgacaagaaccggggcaagagcgacaacgtgccctccgaagaggtcgtgaagaagatgaagaactactggcggcagctgctgaacgccaagctgattacccagagaaagttcgacaatctgaccaaggccgagagaggcggcctgagcgaactggataaggccggcttcatcaagagacagctggtggaaacccggcagatcacaaagcacgtggcacagatcctggactcccggatgaacactaagtacgacgagaatgacaagctgatccgggaagtgaaagtgatcaccctgaagtccaagctggtgtccgatttccggaaggatttccagttttacaaagtgcgcgagatcaacaactaccaccacgcccacgacgcctacctgaacgccgtcgtgggaaccgccctgatcaaaaagtaccctaagctggaaagcgagttcgtgtacggcgactacaaggtgtacgacgtgcggaagatgatcgccaagagcgagcaggaaatcggcaaggctaccgccaagtacttcttctacagcaacatcatgaactttttcaagaccgagattaccctggccaacggcgagatccggaagcggcctctgatcgagacaaacggcgaaaccggggagatcgtgtgggataagggccgggattttgccaccgtgcggaaagtgctgagcatgccccaagtgaatatcgtgaaaaagaccgaggtgcagacaggcggcttcagcaaagagtctatcctgcccaagaggaacagcgataagctgatcgccagaaagaaggactgggaccctaagaagtacggcggcttcgacagccccaccgtggcctattctgtgctggtggtggccaaagtggaaaagggcaagtccaagaaactgaagagtgtgaaagagctgctggggatcaccatcatggaaagaagcagcttcgagaagaatcccatcgactttctggaagccaagggctacaaagaagtgaaaaaggacctgatcatcaagctgcctaagtactccctgttcgagctggaaaacggccggaagagaatgctggcctctgccggcgaactgcagaagggaaacgaactggccctgccctccaaatatgtgaacttcctgtacctggccagccactatgagaagctgaagggctcccccgaggataatgagcagaaacagctgtttgtggaacagcacaagcactacctggacgagatcatcgagcagatcagcgagttctccaagagagtgatcctggccgacgctaatctggacaaagtgctgtccgcctacaacaagcaccgggataagcccatcagagagcaggccgagaatatcatccacctgtttaccctgaccaatctgggagcccctgccgccttcaagtactttgacaccaccatcgaccggaagaggtacaccagcaccaaagaggtgctggacgccaccctgatccaccagagcatcaccggcctgtacgagacacggatcgacctgtctcagctgggaggcgacaaaaggccggcggccacgaaaaaggccggccaggcaaaaaagaaaaagtaagaattcctagagctcgctgatcagcctcgactgtgccttctagttgccagccatctgttgtttgcccctcccccgtgccttccttgaccctggaaggtgccactcccactgtcctttcctaataaaatgaggaaattgcatcgcattgtctgagtaggtgtcattctattctggggggtggggtggggcaggacagcaagggggaggattgggaagagaatagcaggcatgctggggagcggccgcaggaacccctagtgatggagttggccactccctctctgcgcgctcgctcgctcactgaggccgggcgaccaaaggtcgcccgacgcccgggctttgcccgggcggcctcagtgagcgagcgagcgcgcagctgcctgcaggggcgcctgatgcggtattttctccttacgcatctgtgcggtatttcacaccgcatacgtcaaagcaaccatagtacgcgccctgtagcggcgcattaagcgcggcgggtgtggtggttacgcgcagcgtgaccgctacacttgccagcgccctagcgcccgctcctttcgctttcttcccttcctttctcgccacgttcgccggctttccccgtcaagctctaaatcgggggctccctttagggttccgatttagtgctttacggcacctcgaccccaaaaaacttgatttgggtgatggttcacgtagtgggccatcgccctgatagacggtttttcgccctttgacgttggagtccacgttctttaatagtggactcttgttccaaactggaacaacactcaaccctatctcgggctattcttttgatttataagggattttgccgatttcggcctattggttaaaaaatgagctgatttaacaaaaatttaacgcgaattttaacaaaatattaacgtttacaattttatggtgcactctcagtacaatctgctctgatgccgcatagttaagccagccccgacacccgccaacacccgctgacgcgccctgacgggcttgtctgctcccggcatccgcttacagacaagctgtgaccgtctccgggagctgcatgtgtcagaggttttcaccgtcatcaccgaaacgcgcgagacgaaagggcctcgtgatacgcctatttttataggttaatgtcatgataataatggtttcttagacgtcaggtggcacttttcggggaaatgtgcgcggaacccctatttgtttatttttctaaatacattcaaatatgtatccgctcatgagacaataaccctgataaatgcttcaataatattgaaaaaggaagagtatgagtattcaacatttccgtgtcgcccttattcccttttttgcggcattttgccttcctgtttttgctcacccagaaacgctggtgaaagtaaaagatgctgaagatcagttgggtgcacgagtgggttacatcgaactggatctcaacagcggtaagatccttgagagttttcgccccgaagaacgttttccaatgatgagcacttttaaagttctgctatgtggcgcggtattatcccgtattgacgccgggcaagagcaactcggtcgccgcatacactattctcagaatgacttggttgagtactcaccagtcacagaaaagcatcttacggatggcatgacagtaagagaattatgcagtgctgccataaccatgagtgataacactgcggccaacttacttctgacaacgatcggaggaccgaaggagctaaccgcttttttgcacaacatgggggatcatgtaactcgccttgatcgttgggaaccggagctgaatgaagccataccaaacgacgagcgtgacaccacgatgcctgtagcaatggcaacaacgttgcgcaaactattaactggcgaactacttactctagcttcccggcaacaattaatagactggatggaggcggataaagttgcaggaccacttctgcgctcggcccttccggctggctggtttattgctgataaatctggagccggtgagcgtggaagccgcggtatcattgcagcactggggccagatggtaagccctcccgtatcgtagttatctacacgacggggagtcaggcaactatggatgaacgaaatagacagatcgctgagataggtgcctcactgattaagcattggtaactgtcagaccaagtttactcatatatactttagattgatttaaaacttcatttttaatttaaaaggatctaggtgaagatcctttttgataatctc

SEQ ID NO: 6 - DNA, 8508 bp, Artificial Sequence
  Nucleotide sequence of Beta-1,4-N-acetyl galactosaminyl transferase 2-CRISPR/Cas9 vector
atgaccaaaatcccttaacgtgagttttcgttccactgagcgtcagaccccgtagaaaagatcaaaggatcttcttgagatcctttttttctgcgcgtaatctgctgcttgcaaacaaaaaaaccaccgctaccagcggtggtttgtttgccggatcaagagctaccaactctttttccgaaggtaactggcttcagcagagcgcagataccaaatactgtccttctagtgtagccgtagttaggccaccacttcaagaactctgtagcaccgcctacatacctcgctctgctaatcctgttaccagtggctgctgccagtggcgataagtcgtgtcttaccgggttggactcaagacgatagttaccggataaggcgcagcggtcgggctgaacggggggttcgtgcacacagcccagcttggagcgaacgacctacaccgaactgagatacctacagcgtgagctatgagaaagcgccacgcttcccgaagggagaaaggcggacaggtatccggtaagcggcagggtcggaacaggagagcgcacgagggagcttccagggggaaacgcctggtatctttatagtcctgtcgggtttcgccacctctgacttgagcgtcgatttttgtgatgctcgtcaggggggcggagcctatggaaaaacgccagcaacgcggcctttttacggttcctggccttttgctggccttttgctcacatgtgagggcctatttcccatgattccttcatatttgcatatacgatacaaggctgttagagagataattggaattaatttgactgtaaacacaaagatattagtacaaaatacgtgacgtagaaagtaataatttcttgggtagtttgcagttttaaaattatgttttaaaatggactatcatatgcttaccgtaacttgaaagtatttcgatttcttggctttatatatcttgtggaaaggacgaaacaccggtagtactcacgaacactcgttttagagctagaaatagcaagttaaaataaggctagtccgttatcaacttgaaaaagtggcaccgagtcggtgcttttttgttttagagctagaaatagcaagttaaaataaggctagtccgtttttagcgcgtgcgccaattctgcagacaaatggctctagaggtacccgttacataacttacggtaaatggcccgcctggctgaccgcccaacgacccccgcccattgacgtcaatagtaacgccaatagggactttccattgacgtcaatgggtggagtatttacggtaaactgcccacttggcagtacatcaagtgtatcatatgccaagtacgccccctattgacgtcaatgacggtaaatggcccgcctggcattgtgcccagtacatgaccttatgggactttcctacttggcagtacatctacgtattagtcatcgctattaccatggtcgaggtgagccccacgttctgcttcactctccccatctcccccccctccccacccccaattttgtatttatttattttttaattattttgtgcagcgatgggggcggggggggggggggggcgcgcgccaggcggggcggggcggggcgaggggcggggcggggcgaggcggagaggtgcggcggcagccaatcagagcggcgcgctccgaaagtttccttttatggcgaggcggcggcggcggcggccctataaaaagcgaagcgcgcggcgggcgggagtcgctgcgacgctgccttcgccccgtgccccgctccgccgccgcctcgcgccgcccgccccggctctgactgaccgcgttactcccacaggtgagcgggcgggacggcccttctcctccgggctgtaattagctgagcaagaggtaagggtttaagggatggttggttggtggggtattaatgtttaattacctggagcacctgcctgaaatcactttttttcaggttggaccggtgccaccatggactataaggaccacgacggagactacaaggatcatgatattgattacaaagacgatgacgataagatggccccaaagaagaagcggaaggtcggtatccacggagtcccagcagccgacaagaagtacagcatcggcctggacatcggcaccaactctgtgggctgggccgtgatcaccgacgagtacaaggtgcccagcaagaaattcaaggtgctgggcaacaccgaccggcacagcatcaagaagaacctgatcggagccctgctgttcgacagcggcgaaacagccgaggccacccggctgaagagaaccgccagaagaagatacaccagacggaagaaccggatctgctatctgcaagagatcttcagcaacgagatggccaaggtggacgacagcttcttccacagactggaagagtccttcctggtggaagaggataagaagcacgagcggcaccccatcttcggcaacatcgtggacgaggtggcctaccacgagaagtaccccaccatctaccacctgagaaagaaactggtggacagcaccgacaaggccgacctgcggctgatctatctggccctggcccacatgatcaagttccggggccacttcctgatcgagggcgacctgaaccccgacaacagcgacgtggacaagctgttcatccagctggtgcagacctacaaccagctgttcgaggaaaaccccatcaacgccagcggcgtggacgccaaggccatcctgtctgccagactgagcaagagcagacggctggaaaatctgatcgcccagctgcccggcgagaagaagaatggcctgttcggaaacctgattgccctgagcctgggcctgacccccaacttcaagagcaacttcgacctggccgaggatgccaaactgcagctgagcaaggacacctacgacgacgacctggacaacctgctggcccagatcggcgaccagtacgccgacctgtttctggccgccaagaacctgtccgacgccatcctgctgagcgacatcctgagagtgaacaccgagatcaccaaggcccccctgagcgcctctatgatcaagagatacgacgagcaccaccaggacctgaccctgctgaaagctctcgtgcggcagcagctgcctgagaagtacaaagagattttcttcgaccagagcaagaacggctacgccggctacattgacggcggagccagccaggaagagttctacaagttcatcaagcccatcctggaaaagatggacggcaccgaggaactgctcgtgaagctgaacagagaggacctgctgcggaagcagcggaccttcgacaacggcagcatcccccaccagatccacctgggagagctgcacgccattctgcggcggcaggaagatttttacccattcctgaaggacaaccgggaaaagatcgagaagatcctgaccttccgcatcccctactacgtgggccctctggccaggggaaacagcagattcgcctggatgaccagaaagagcgaggaaaccatcaccccctggaacttcgaggaagtggtggacaagggcgcttccgcccagagcttcatcgagcggatgaccaacttcgataagaacctgcccaacgagaaggtgctgcccaagcacagcctgctgtacgagtacttcaccgtgtataacgagctgaccaaagtgaaatacgtgaccgagggaatgagaaagcccgccttcctgagcggcgagcagaaaaaggccatcgtggacctgctgttcaagaccaaccggaaagtgaccgtgaagcagctgaaagaggactacttcaagaaaatcgagtgcttcgactccgtggaaatctccggcgtggaagatcggttcaacgcctccctgggcacataccacgatctgctgaaaattatcaaggacaaggacttcctggacaatgaggaaaacgaggacattctggaagatatcgtgctgaccctgacactgtttgaggacagagagatgatcgaggaacggctgaaaacctatgcccacctgttcgacgacaaagtgatgaagcagctgaagcggcggagatacaccggctggggcaggctgagccggaagctgatcaacggcatccgggacaagcagtccggcaagacaatcctggatttcctgaagtccgacggcttcgccaacagaaacttcatgcagctgatccacgacgacagcctgacctttaaagaggacatccagaaagcccaggtgtccggccagggcgatagcctgcacgagcacattgccaatctggccggcagccccgccattaagaagggcatcctgcagacagtgaaggtggtggacgagctcgtgaaagtgatgggccggcacaagcccgagaacatcgtgatcgaaatggccagagagaaccagaccacccagaagggacagaagaacagccgcgagagaatgaagcggatcgaagagggcatcaaagagctgggcagccagatcctgaaagaacaccccgtggaaaacacccagctgcagaacgagaagctgtacctgtactacctgcagaatgggcgggatatgtacgtggaccaggaactggacatcaaccggctgtccgactacgatgtggaccatatcgtgcctcagagctttctgaaggacgactccatcgacaacaaggtgctgaccagaagcgacaagaaccggggcaagagcgacaacgtgccctccgaagaggtcgtgaagaagatgaagaactactggcggcagctgctgaacgccaagctgattacccagagaaagttcgacaatctgaccaaggccgagagaggcggcctgagcgaactggataaggccggcttcatcaagagacagctggtggaaacccggcagatcacaaagcacgtggcacagatcctggactcccggatgaacactaagtacgacgagaatgacaagctgatccgggaagtgaaagtgatcaccctgaagtccaagctggtgtccgatttccggaaggatttccagttttacaaagtgcgcgagatcaacaactaccaccacgcccacgacgcctacctgaacgccgtcgtgggaaccgccctgatcaaaaagtaccctaagctggaaagcgagttcgtgtacggcgactacaaggtgtacgacgtgcggaagatgatcgccaagagcgagcaggaaatcggcaaggctaccgccaagtacttcttctacagcaacatcatgaactttttcaagaccgagattaccctggccaacggcgagatccggaagcggcctctgatcgagacaaacggcgaaaccggggagatcgtgtgggataagggccgggattttgccaccgtgcggaaagtgctgagcatgccccaagtgaatatcgtgaaaaagaccgaggtgcagacaggcggcttcagcaaagagtctatcctgcccaagaggaacagcgataagctgatcgccagaaagaaggactgggaccctaagaagtacggcggcttcgacagccccaccgtggcctattctgtgctggtggtggccaaagtggaaaagggcaagtccaagaaactgaagagtgtgaaagagctgctggggatcaccatcatggaaagaagcagcttcgagaagaatcccatcgactttctggaagccaagggctacaaagaagtgaaaaaggacctgatcatcaagctgcctaagtactccctgttcgagctggaaaacggccggaagagaatgctggcctctgccggcgaactgcagaagggaaacgaactggccctgccctccaaatatgtgaacttcctgtacctggccagccactatgagaagctgaagggctcccccgaggataatgagcagaaacagctgtttgtggaacagcacaagcactacctggacgagatcatcgagcagatcagcgagttctccaagagagtgatcctggccgacgctaatctggacaaagtgctgtccgcctacaacaagcaccgggataagcccatcagagagcaggccgagaatatcatccacctgtttaccctgaccaatctgggagcccctgccgccttcaagtactttgacaccaccatcgaccggaagaggtacaccagcaccaaagaggtgctggacgccaccctgatccaccagagcatcaccggcctgtacgagacacggatcgacctgtctcagctgggaggcgacaaaaggccggcggccacgaaaaaggccggccaggcaaaaaagaaaaagtaagaattcctagagctcgctgatcagcctcgactgtgccttctagttgccagccatctgttgtttgcccctcccccgtgccttccttgaccctggaaggtgccactcccactgtcctttcctaataaaatgaggaaattgcatcgcattgtctgagtaggtgtcattctattctggggggtggggtggggcaggacagcaagggggaggattgggaagagaatagcaggcatgctggggagcggccgcaggaacccctagtgatggagttggccactccctctctgcgcgctcgctcgctcactgaggccgggcgaccaaaggtcgcccgacgcccgggctttgcccgggcggcctcagtgagcgagcgagcgcgcagctgcctgcaggggcgcctgatgcggtattttctccttacgcatctgtgcggtatttcacaccgcatacgtcaaagcaaccatagtacgcgccctgtagcggcgcattaagcgcggcgggtgtggtggttacgcgcagcgtgaccgctacacttgccagcgccctagcgcccgctcctttcgctttcttcccttcctttctcgccacgttcgccggctttccccgtcaagctctaaatcgggggctccctttagggttccgatttagtgctttacggcacctcgaccccaaaaaacttgatttgggtgatggttcacgtagtgggccatcgccctgatagacggtttttcgccctttgacgttggagtccacgttctttaatagtggactcttgttccaaactggaacaacactcaaccctatctcgggctattcttttgatttataagggattttgccgatttcggcctattggttaaaaaatgagctgatttaacaaaaatttaacgcgaattttaacaaaatattaacgtttacaattttatggtgcactctcagtacaatctgctctgatgccgcatagttaagccagccccgacacccgccaacacccgctgacgcgccctgacgggcttgtctgctcccggcatccgcttacagacaagctgtgaccgtctccgggagctgcatgtgtcagaggttttcaccgtcatcaccgaaacgcgcgagacgaaagggcctcgtgatacgcctatttttataggttaatgtcatgataataatggtttcttagacgtcaggtggcacttttcggggaaatgtgcgcggaacccctatttgtttatttttctaaatacattcaaatatgtatccgctcatgagacaataaccctgataaatgcttcaataatattgaaaaaggaagagtatgagtattcaacatttccgtgtcgcccttattcccttttttgcggcattttgccttcctgtttttgctcacccagaaacgctggtgaaagtaaaagatgctgaagatcagttgggtgcacgagtgggttacatcgaactggatctcaacagcggtaagatccttgagagttttcgccccgaagaacgttttccaatgatgagcacttttaaagttctgctatgtggcgcggtattatcccgtattgacgccgggcaagagcaactcggtcgccgcatacactattctcagaatgacttggttgagtactcaccagtcacagaaaagcatcttacggatggcatgacagtaagagaattatgcagtgctgccataaccatgagtgataacactgcggccaacttacttctgacaacgatcggaggaccgaaggagctaaccgcttttttgcacaacatgggggatcatgtaactcgccttgatcgttgggaaccggagctgaatgaagccataccaaacgacgagcgtgacaccacgatgcctgtagcaatggcaacaacgttgcgcaaactattaactggcgaactacttactctagcttcccggcaacaattaatagactggatggaggcggataaagttgcaggaccacttctgcgctcggcccttccggctggctggtttattgctgataaatctggagccggtgagcgtggaagccgcggtatcattgcagcactggggccagatggtaagccctcccgtatcgtagttatctacacgacggggagtcaggcaactatggatgaacgaaatagacagatcgctgagataggtgcctcactgattaagcattggtaactgtcagaccaagtttactcatatatactttagattgatttaaaacttcatttttaatttaaaaggatctaggtgaagatcctttttgataatctc

SEQ ID NO: 7 - DNA, 22 bp, Artificial Sequence
  SgRNA forward primer of GGTA1 gene
caccgaaaataatgaatgtcaa

SEQ ID NO: 8 - DNA, 22 bp, Artificial Sequence
  SgRNA reverse primer of GGTA1 gene
aaacttgacattcattattttc

SEQ ID NO: 9 - DNA, 25 bp, Artificial Sequence
  SgRNA forward primer of CMAH gene
caccggagtaaggtacgtgatctgt

SEQ ID NO: 10 - DNA, 25 bp, Artificial Sequence
  SgRNA reverse primer of CMAH gene
aaacacagatcacgtaccttactcc

SEQ ID NO: 11 - DNA, 24 bp, Artificial Sequence
  SgRNA forward primer of Beta-1,4-N-acetyl galactosaminyl transferase 2 gene
caccggtagtactcacgaacactc

SEQ ID NO: 12 - DNA, 24 bp, Artificial Sequence
  SgRNA reverse primer of Beta-1,4-N-acetyl galactosaminyl transferase 2 gene
aaacgagtgttcgtgagtactacc

SEQ ID NO: 13 - DNA, 25 bp, Artificial Sequence
  Forward primer of GGTA1 gene
ccttagtatccttcccaacccagac

SEQ ID NO: 14 - DNA, 26 bp, Artificial Sequence
  Reverse primer of GGTA1 gene
gctttctttacggtgtcagtgaatcc

SEQ ID NO: 15 - DNA, 22 bp, Artificial Sequence
  Forward primer of CMAH gene
cttggaggtgatttgagttggg

SEQ ID NO: 16 - DNA, 22 bp, Artificial Sequence
  Reverse primer of CMAH gene
cattttcttcggagttgagggc

SEQ ID NO: 17 - DNA, 18 bp, Artificial Sequence
  Forward primer of Beta-1,4-N-acetyl galactosaminyl transferase 2 gene
cccaaggatcctgctgcc

SEQ ID NO: 18 - DNA, 20 bp, Artificial Sequence
  Reverse primer of Beta-1,4-N-acetyl galactosaminyl transferase 2 gene
cgccgtgtaaagaaacctcc

SEQ ID NO: 19 - DNA, 47 bp, Sus scrofa
ttttcccaggagaaaataatgaatgtcaaaggaagagtggttctgtc

SEQ ID NO: 20 - DNA, 47 bp, Sus scrofa
aggtccatgcaggcgtgagtaaggtacgtgatctgttggaagacagt

SEQ ID NO: 21 - DNA, 47 bp, Sus scrofa
gggtagtactcacgaacactccggagcatggtcatgagcttgtgggg